European Patent Specification EP 3 529 622 B1, published March 12, 2025. Title: GENETICALLY ENCODED CELL DEATH INDICATORS AND METHODS OF USE. Applicant: THE J. DAVID GLADSTONE INSTITUTES LINSLEY, Jeremy SHAH, Kevan FINKBEINER, Steven M. The sequence listing filed with the application follows.

SEQUENCE LISTING (12 sequences)

SEQ ID NO: 1 - DNA, 1353 bp, Artificial Sequence
  GCaMP
atgggttctcatcatcatcatcatcatggtatggctagcatgactggtggacagcaaatgggtcgggatctgtacgacgatgacgataaggatctcgccaccatggtcgactcatcacgtcgtaagtggaataagacaggtcacgcagtcagagctataggtcggctgagctcactcgagaacgtctatatcaaggccgacaagcagaagaacggcatcaaggcgaacttcaagatccgccacaacatcgaggacggcggcgtgcagctcgcctaccactaccagcagaacacccccatcggcgacggccccgtgctgctgcccgacaaccactacctgagcgtgcagtccaaactttcgaaagaccccaacgagaagcgcgatcacatggtcctgctggagttcgtgaccgccgccgggatcactctcggcatggacgagctgtacaagggcggtaccggagggagcatggtgagcaagggcgaggagctgttcaccggggtggtgcccatcctggtcgagctggacggcgacgtaaacggccacaagttcagcgtgtccggcgagggtgagggcgatgccacctacggcaagctgaccctgaagttcatctgcaccaccggcaagctgcccgtgccctggcccaccctcgtgaccaccctgacctacggcgtgcagtgcttcagccgctaccccgaccacatgaagcagcacgacttcttcaagtccgccatgcccgaaggctacatccaggagcgcaccatcttcttcaaggacgacggcaactacaagacccgcgccgaggtgaagttcgagggcgacaccctggtgaaccgcatcgagctgaagggcatcgacttcaaggaggacggcaacatcctggggcacaagctggagtacaacctgccggaccaactgactgaagagcagatcgcagaatttaaagaggaattctccctatttgacaaggacggggatgggacaataacaaccaaggagctggggacggtgatgcggtctctggggcagaaccccacagaagcagagctgcaggacatgatcaatgaagtagatgccgacggtgacggcacaatcgacttccctgagttcctgacaatgatggcaagaaaaatgaaatacagggacacggaagaagaaattagagaagcgttcggtgtgtttgataaggatggcaatggctacatcagtgcagcagagcttcgccacgtgatgacaaaccttggagagaagttaacagatgaagaggttgatgaaatgatcagggaagcagacatcgatggggatggtcaggtaaactacgaagagtttgtacaaatgatgacagcgaagtga

SEQ ID NO: 2 - DNA, 1251 bp, Artificial Sequence
  CEPIA - Suzuki
atggtcgactcttcacgtcgtaagtggaataagacaggtcacgcagtcagagctataggtcggctgagctcaccagagaacgtgtatataaaggccgacgagcagaagaacggcatcaaggcgtacttcaagatccgccacaacatcgagggcggcggcgtgcagctcgcctaccactaccagcagatcacccccataggcgacggccccgtgctgctgcccgacaaccactacctgagcgtgcagtccatactttcgaaagaccccaacgagaagcgcgatcacatggtcctgctggagttcgtgaccgccgccgggatcactctcggcatggacgagctgtacaagggtggcagcggtggcatggtgagcaagggcgaggagctgttcaccggggtggtgcccatccaggtcgagctggacggcgacgtaaacggccacaagttcagcgtgtccggcgagggtgagggcgatgccacctacggcaagctgaccctgaagttcatctgcaccaccggcaagctgcccgtgccctggcccaccctcgtgaccaccctgtcctacggcgtgcagtgcttcagccgctaccccgaccacatgaagcagcacgacttcttcaagtccgccatgcccgaaggctacatccaggagcgcaccatcttcttcaaggacgacggcaactacaagacccgcgccgaggtgaagttcgagggcgacaccctggtgaaccgcatcgagctgaagggcatcgacttcaaggaggacggcaacatcctggggcacaagctggagtacagcacgcgtgaccaactgactgaagagcagatcgcagaatttaaagaggctttctccctatttgacaaggacggggatgggacgataacaaccaaggatctggggacggtgatgcggtctctggggcagaaccccacagaagcagagctccaggacatgatcaatgaagtagatgccgacggtgacggcacaatcgacttccctgagttcctgacaatgatggcacctaaaatgcaggacacagacagtgaagaggaaattcgcgaagcgttccgtgtgtgggataaggatggcaatggctacatcggcgcagcagagcttcgccacgtgatgacaaaccttggagagaagttaacagatgaagaggttgatgaaatgatcagggtagcagacatcgatggagaaggtcaggtaaactacgaagactttgtacaaatgatgacagcgaaggcggcc

SEQ ID NO: 3 - protein, 450 aa, Artificial Sequence
  GCaMP
MGSHHHHHHGMASMTGGQQMGRDLYDDDDKDLATMVDSSRRKWNKTGHAVRAIGRLSSLENVYIKADKQKNGIKANFKIRHNIEDGGVQLAYHYQQNTPIGDGPVLLPDNHYLSVQSKLSKDPNEKRDHMVLLEFVTAAGITLGMDELYKGGTGGSMVSKGEELFTGVVPILVELDGDVNGHKFSVSGEGEGDATYGKLTLKFICTTGKLPVPWPTLVTTLTYGVQCFSRYPDHMKQHDFFKSAMPEGYIQERTIFFKDDGNYKTRAEVKFEGDTLVNRIELKGIDFKEDGNILGHKLEYNTRDQLTEEQIAEFKEAFSLFDKDGDGTITTKELGTVMRSLGQNPTEAELQDMINEVDADGDGTIDFPEFLTMMARKMKDTDSEEEIREAFRVFDKDGNGYISAAELRHVMTNLGEKLTDEEVDEMIREADIDGDGQVNYEEFVQMMTAK

SEQ ID NO: 4 - protein, 417 aa, Artificial Sequence
  CEPIA Sequence - Suzuki
MVDSSRRKWNKTGHAVRAIGRLSSPENVYIKADEQKNGIKAYFKIRHNIEGGGVQLAYHYQQITPIGDGPVLLPDNHYLSVQSILSKDPNEKRDHMVLLEFVTAAGITLGMDELYKGGSGGMVSKGEELFTGVVPIQVELDGDVNGHKFSVSGEGEGDATYGKLTLKFICTTGKLPVPWPTLVTTLSYGVQCFSRYPDHMKQHDFFKSAMPEGYIQERTIFFKDDGNYKTRAEVKFEGDTLVNRIELKGIDFKEDGNILGHKLEYSTRDQLTEEQIAEFKEAFSLFDKDGDGTITTKDLGTVMRSLGQNPTEAELQDMINEVDADGDGTIDFPEFLTMMAPKMQDTDSEEEIREAFRVWDKDGNGYIGAAELRHVMTNLGEKLTDEEVDEMIRVADIDGEGQVNYEDFVQMMTAKAA

SEQ ID NO: 5 - protein, 148 aa, Artificial Sequence
  Calmodulin
ADQLTEEQIAEFKEAFSLFDKDGDGTITTKELGTVMRSLGQNPTEAELQDMINEVDADGNGTIDFPEFLTMMARKMKDTDSEEEIREAFRVFDKDGNGYISAAELRHVMTNLGEKLTDEEVDEMIREADIDGDGQVNYEEFVQMMTAK

SEQ ID NO: 6 - DNA, 6213 bp, Artificial Sequence
  Hsyn1:RGEDI-P2a-EGFP
ctaaattgtaagcgttaatattttgttaaaattcgcgttaaatttttgttaaatcagctcattttttaaccaataggccgaaatcggcaaaatcccttataaatcaaaagaatagaccgagatagggttgagtgttgttccagtttggaacaagagtccactattaaagaacgtggactccaacgtcaaagggcgaaaaaccgtctatcagggcgatggcccactacgtgaaccatcaccctaatcaagttttttggggtcgaggtgccgtaaagcactaaatcggaaccctaaagggagcccccgatttagagcttgacggggaaagccggcgaacgtggcgagaaaggaagggaagaaagcgaaaggagcgggcgctagggcgctggcaagtgtagcggtcacgctgcgcgtaaccaccacacccgccgcgcttaatgcgccgctacagggcgcgtcccattcgccattcaggctgcgcaactgttgggaagggcgatcggtgcgggcctcttcgctattacgccagctggcgaaagggggatgtgctgcaaggcgattaagttgggtaacgccagggttttcccagtcacgacgttgtaaaacgacggccagtgagcgcgcgtaatacgactcactatagggcgaattgggtaccgggctgcagagggccctgcgtatgagtgcaagtgggttttaggaccaggatgaggcggggtgggggtgcctacctgacgaccgaccccgacccactggacaagcacccaacccccattccccaaattgcgcatcccctatcagagagggggaggggaaacaggatgcggcgaggcgcgtgcgcactgccagcttcagcaccgcggacagtgccttcgcccccgcctggcggcgcgcgccaccgccgcctcagcactgaaggcgcgctgacgtcactcgccggtcccccgcaaactccccttcccggccaccttggtcgcgtccgcgccgccgccggcccagccggaccgcaccacgcgaggcgcgagataggggggcacgggcgcgaccatctgcgctgcggcgccggcgactcagcgctgcctcagtctgcggtgggcagcggaggagtcgtgtcgtgcctgagagcgcagtcgaattcaagctgctagctagtaccggtcctagggccccccccctcgaggtcgacggtatcgataagcttgccgccaccatgggtgacaatgacatccactttgcctttctctccacaggcgcgcactcccaggtccaactgcagggatccatggtcgactcttcacgtcgtaagtggaataaggcaggtcacgcagtcagagctataggtcggctgagctcacccgtggtttccgagcggatgtaccccgaggacggcgccctgaagagcgagatcaagaaggggctgaggctgaaggacggcggccactacgccgccgaggtcaagaccacctacaaggccaagaagcccgtgcagctgcccggcgcctacatcgtcgacatcaagttggacatcgtgtcccacaacgaggactacaccatcgtggaacagtgcgaacgcgccgagggccgccactccaccggcggcatggacgagctgtacaagggaggtacaggcgggagtctggtgagcaagggcgaggaggataacatggccatcatcaaggagttcatgcgcttcaaggtgcacatggagggctccgtgaacggccacgagttcgagatcgagggcgagggcgagggccgcccctacgaggcctttcagaccgctaagctgaaggtgaccaagggtggccccctgcccttcgcctgggacatcctgtcccctcagttcatgtacggctccaaggcctacattaagcacccagccgacatccccgactacttcaagctgtccttccccgagggcttcaggtgggagcgcgtgatgaacttcgaggacggcggcattattcacgttaaccaggactcctccctgcaggacggcgtattcatctacaaggtgaagctgcgcggcaccaacttcccccccgacggccccgtaatgcagaagaagaccatgggctgggaggctactcgagaccaactgactgaagagcagatcgcagaatttaaagaggctttctccctatttgacaaggacggggatgggacaataacaaccaaggatctggggacggtgctgcggtctctggggcagaaccccacagaagcagagctccaggacatgatcaatgaagtagatgccgacggtaatggcacaatcgacttccctgatttcctgacaatgatggcaagaaaaatgaaagacacagacagtgaagaagaaattcgcgaagcgttccgtgtgtgggataaggatggcaatggctacatctctgcagcagaccttcgccacgtgatgacaaaccttggagagaagttaacagatgaagaggttgatgaaatgatcagggaagcagatatcgatggagaaggtcaggtaaactacgaagagtttgtacaaatgatgacagcgaaggcggccgcagaacaaaaactcatctcagaagaggatctgaatggggccgcaagcgagggatccggatccggagccacgaacttctctctgttaaagcaagcaggagacgtggaagaaaaccccggtcctatggtgagcaagggcgaggagctgttcaccggggtggtgcccatcctggtcgagctggacggcgacgtaaacggccacaagttcagcgtgtccggcgagggcgagggcgatgccacctacggcaagctgaccctgaagttcatctgcaccaccggcaagctgcccgtgccctggcccaccctcgtgaccaccctgacctacggcgtgcagtgcttcagccgctaccccgaccacatgaagcagcacgacttcttcaagtccgccatgcccgaaggctacgtccaggagcgcaccatcttcttcaaggacgacggcaactacaagacccgcgccgaggtgaagttcgagggcgacaccctggtgaaccgcatcgagctgaagggcatcgacttcaaggaggacggcaacatcctggggcacaagctggagtacaactacaacagccacaacgtctatatcatggccgacaagcagaagaacggcatcaaggtgaacttcaagatccgccacaacatcgaggacggcagcgtgcagctcgccgaccactaccagcagaacacccccatcggcgacggccccgtgctgctgcccgacaaccactacctgagcacccagtccgccctgagcaaagaccccaacgagaagcgcgatcacatggtcctgctggagttcgtgaccgccgccgggatcactctcggcatggacgagctgtacaagtaaactagttctagagcggccgccaccgcggtgtcgataatcaacctctggattacaaaatttgtgaaagattgactggtattcttaactatgttgctccttttacgctatgtggatacgctgctttaatgcctttgtatcatgctattgcttcccgtatggctttcattttctcctccttgtataaatcctggttgctgtctctttatgaggagttgtggcccgttgtcaggcaacgtggcgtggtgtgcactgtgtttgctgacgcaacccccactggttggggcattgccaccacctgtcagctcctttccgggactttcgctttccccctccctattgccacggcggaactcatcgccgcctgccttgcccgctgctggacaggggctcggctgttgggcactgacaattccgtggtgttgtcggggaaatcatcgtcctttccttggctgctcgcctgtgttgccacctggattctgcgcgggacgtccttctgctacgtcccttcggccctcaatccagcggaccttccttcccgcggcctgctgccggctctgcggcctcttccgcgtcttcgccttcgccctcagacgagtcggatctccctttgggccgcctccccgcgagctccagcttttgttccctttagtgagggttaattgcgcgcttggcgtaatcatggtcatagctgtttcctgtgtgaaattgttatccgctcacaattccacacaacatacgagccggaagcataaagtgtaaagcctggggtgcctaatgagtgagctaactcacattaattgcgttgcgctcactgcccgctttccagtcgggaaacctgtcgtgccagctgcattaatgaatcggccaacgcgcggggagaggcggtttgcgtattgggcgctcttccgcttcctcgctcactgactcgctgcgctcggtcgttcggctgcggcgagcggtatcagctcactcaaaggcggtaatacggttatccacagaatcaggggataacgcaggaaagaacatgtgagcaaaaggccagcaaaaggccaggaaccgtaaaaaggccgcgttgctggcgtttttccataggctccgcccccctgacgagcatcacaaaaatcgacgctcaagtcagaggtggcgaaacccgacaggactataaagataccaggcgtttccccctggaagctccctcgtgcgctctcctgttccgaccctgccgcttaccggatacctgtccgcctttctcccttcgggaagcgtggcgctttctcatagctcacgctgtaggtatctcagttcggtgtaggtcgttcgctccaagctgggctgtgtgcacgaaccccccgttcagcccgaccgctgcgccttatccggtaactatcgtcttgagtccaacccggtaagacacgacttatcgccactggcagcagccactggtaacaggattagcagagcgaggtatgtaggcggtgctacagagttcttgaagtggtggcctaactacggctacactagaaggacagtatttggtatctgcgctctgctgaagccagttaccttcggaaaaagagttggtagctcttgatccggcaaacaaaccaccgctggtagcggtggtttttttgtttgcaagcagcagattacgcgcagaaaaaaaggatctcaagaagatcctttgatcttttctacggggtctgacgctcagtggaacgaaaactcacgttaagggattttggtcatgagattatcaaaaaggatcttcacctagatccttttaaattaaaaatgaagttttaaatcaatctaaagtatatatgagtaaacttggtctgacagttaccaatgcttaatcagtgaggcacctatctcagcgatctgtctatttcgttcatccatagttgcctgactccccgtcgtgtagataactacgatacgggagggcttaccatctggccccagtgctgcaatgataccgcgagacccacgctcaccggctccagatttatcagcaataaaccagccagccggaagggccgagcgcagaagtggtcctgcaactttatccgcctccatccagtctattaattgttgccgggaagctagagtaagtagttcgccagttaatagtttgcgcaacgttgttgccattgctacaggcatcgtggtgtcacgctcgtcgtttggtatggcttcattcagctccggttcccaacgatcaaggcgagttacatgatcccccatgttgtgcaaaaaagcggttagctccttcggtcctccgatcgttgtcagaagtaagttggccgcagtgttatcactcatggttatggcagcactgcataattctcttactgtcatgccatccgtaagatgcttttctgtgactggtgagtactcaaccaagtcattctgagaatagtgtatgcggcgaccgagttgctcttgcccggcgtcaatacgggataataccgcgccacatagcagaactttaaaagtgctcatcattggaaaacgttcttcggggcgaaaactctcaaggatcttaccgctgttgagatccagttcgatgtaacccactcgtgcacccaactgatcttcagcatcttttactttcaccagcgtttctgggtgagcaaaaacaggaaggcaaaatgccgcaaaaaagggaataagggcgacacggaaatgttgaatactcatactcttcctttttcaatattattgaagcatttatcagggttattgtctcatgagcggatacatatttgaatgtatttagaaaaataaacaaataggggttccgcgcacatttccccgaaaagtgccac

SEQ ID NO: 7 - DNA, 6228 bp, Artificial Sequence
  Hsyn1:RGEDI-P2a-TagBFP2
ctaaattgtaagcgttaatattttgttaaaattcgcgttaaatttttgttaaatcagctcattttttaaccaataggccgaaatcggcaaaatcccttataaatcaaaagaatagaccgagatagggttgagtgttgttccagtttggaacaagagtccactattaaagaacgtggactccaacgtcaaagggcgaaaaaccgtctatcagggcgatggcccactacgtgaaccatcaccctaatcaagttttttggggtcgaggtgccgtaaagcactaaatcggaaccctaaagggagcccccgatttagagcttgacggggaaagccggcgaacgtggcgagaaaggaagggaagaaagcgaaaggagcgggcgctagggcgctggcaagtgtagcggtcacgctgcgcgtaaccaccacacccgccgcgcttaatgcgccgctacagggcgcgtcccattcgccattcaggctgcgcaactgttgggaagggcgatcggtgcgggcctcttcgctattacgccagctggcgaaagggggatgtgctgcaaggcgattaagttgggtaacgccagggttttcccagtcacgacgttgtaaaacgacggccagtgagcgcgcgtaatacgactcactatagggcgaattgggtaccgggctgcagagggccctgcgtatgagtgcaagtgggttttaggaccaggatgaggcggggtgggggtgcctacctgacgaccgaccccgacccactggacaagcacccaacccccattccccaaattgcgcatcccctatcagagagggggaggggaaacaggatgcggcgaggcgcgtgcgcactgccagcttcagcaccgcggacagtgccttcgcccccgcctggcggcgcgcgccaccgccgcctcagcactgaaggcgcgctgacgtcactcgccggtcccccgcaaactccccttcccggccaccttggtcgcgtccgcgccgccgccggcccagccggaccgcaccacgcgaggcgcgagataggggggcacgggcgcgaccatctgcgctgcggcgccggcgactcagcgctgcctcagtctgcggtgggcagcggaggagtcgtgtcgtgcctgagagcgcagtcgaattcaagctgctagctagtaccggtcctagggccccccccctcgaggtcgacggtatcgataagcttgccgccaccatgggtgacaatgacatccactttgcctttctctccacaggcgcgcactcccaggtccaactgcagggatccatggtcgactcttcacgtcgtaagtggaataaggcaggtcacgcagtcagagctataggtcggctgagctcacccgtggtttccgagcggatgtaccccgaggacggcgccctgaagagcgagatcaagaaggggctgaggctgaaggacggcggccactacgccgccgaggtcaagaccacctacaaggccaagaagcccgtgcagctgcccggcgcctacatcgtcgacatcaagttggacatcgtgtcccacaacgaggactacaccatcgtggaacagtgcgaacgcgccgagggccgccactccaccggcggcatggacgagctgtacaagggaggtacaggcgggagtctggtgagcaagggcgaggaggataacatggccatcatcaaggagttcatgcgcttcaaggtgcacatggagggctccgtgaacggccacgagttcgagatcgagggcgagggcgagggccgcccctacgaggcctttcagaccgctaagctgaaggtgaccaagggtggccccctgcccttcgcctgggacatcctgtcccctcagttcatgtacggctccaaggcctacattaagcacccagccgacatccccgactacttcaagctgtccttccccgagggcttcaggtgggagcgcgtgatgaacttcgaggacggcggcattattcacgttaaccaggactcctccctgcaggacggcgtattcatctacaaggtgaagctgcgcggcaccaacttcccccccgacggccccgtaatgcagaagaagaccatgggctgggaggctactcgagaccaactgactgaagagcagatcgcagaatttaaagaggctttctccctatttgacaaggacggggatgggacaataacaaccaaggatctggggacggtgctgcggtctctggggcagaaccccacagaagcagagctccaggacatgatcaatgaagtagatgccgacggtaatggcacaatcgacttccctgatttcctgacaatgatggcaagaaaaatgaaagacacagacagtgaagaagaaattcgcgaagcgttccgtgtgtgggataaggatggcaatggctacatctctgcagcagaccttcgccacgtgatgacaaaccttggagagaagttaacagatgaagaggttgatgaaatgatcagggaagcagatatcgatggagaaggtcaggtaaactacgaagagtttgtacaaatgatgacagcgaaggcggccgcagaacaaaaactcatctcagaagaggatctgaatggggccgcaagcgagggatccggatccggagccacgaacttctctctgttaaagcaagcaggagacgtggaagaaaaccccggtcctgggagccaccatcaccatcaccatggcagatctatgagcgagctgattaaggagaacatgcacatgaagctgtacatggagggcaccgtggacaaccatcacttcaagtgcacatccgagggcgaaggcaagccctacgagggcacccagaccatgagaatcaaggtggtcgagggcggccctctccccttcgccttcgacatcctggctactagcttcctctacggcagcaagaccttcatcaaccacacccagggcatccccgacttcttcaagcagtccttccctgagggcttcacatgggagagagtcaccacatacgaagacgggggcgtgctgaccgctacccaggacaccagcctccaggacggctgcctcatctacaacgtcaagatcagaggggtgaacttcacatccaacggccctgtgatgcagaagaaaacactcggctgggaggccttcaccgagacgctgtaccccgctgacggcggcctggaaggcagaaacgacatggccctgaagctcgtgggcgggagccatctgatcgcaaacgccaagaccacatatagatccaagaaacccgctaagaacctcaagatgcctggcgtctactatgtggactacagactggaaagaatcaaggaggccaacaacgagacctacgtcgagcagcacgaggtggcagtggccagatactgcgacctccctagcaaactggggcacaagcttaattaaactagttctagagcggccgccaccgcggtgtcgataatcaacctctggattacaaaatttgtgaaagattgactggtattcttaactatgttgctccttttacgctatgtggatacgctgctttaatgcctttgtatcatgctattgcttcccgtatggctttcattttctcctccttgtataaatcctggttgctgtctctttatgaggagttgtggcccgttgtcaggcaacgtggcgtggtgtgcactgtgtttgctgacgcaacccccactggttggggcattgccaccacctgtcagctcctttccgggactttcgctttccccctccctattgccacggcggaactcatcgccgcctgccttgcccgctgctggacaggggctcggctgttgggcactgacaattccgtggtgttgtcggggaaatcatcgtcctttccttggctgctcgcctgtgttgccacctggattctgcgcgggacgtccttctgctacgtcccttcggccctcaatccagcggaccttccttcccgcggcctgctgccggctctgcggcctcttccgcgtcttcgccttcgccctcagacgagtcggatctccctttgggccgcctccccgcgagctccagcttttgttccctttagtgagggttaattgcgcgcttggcgtaatcatggtcatagctgtttcctgtgtgaaattgttatccgctcacaattccacacaacatacgagccggaagcataaagtgtaaagcctggggtgcctaatgagtgagctaactcacattaattgcgttgcgctcactgcccgctttccagtcgggaaacctgtcgtgccagctgcattaatgaatcggccaacgcgcggggagaggcggtttgcgtattgggcgctcttccgcttcctcgctcactgactcgctgcgctcggtcgttcggctgcggcgagcggtatcagctcactcaaaggcggtaatacggttatccacagaatcaggggataacgcaggaaagaacatgtgagcaaaaggccagcaaaaggccaggaaccgtaaaaaggccgcgttgctggcgtttttccataggctccgcccccctgacgagcatcacaaaaatcgacgctcaagtcagaggtggcgaaacccgacaggactataaagataccaggcgtttccccctggaagctccctcgtgcgctctcctgttccgaccctgccgcttaccggatacctgtccgcctttctcccttcgggaagcgtggcgctttctcatagctcacgctgtaggtatctcagttcggtgtaggtcgttcgctccaagctgggctgtgtgcacgaaccccccgttcagcccgaccgctgcgccttatccggtaactatcgtcttgagtccaacccggtaagacacgacttatcgccactggcagcagccactggtaacaggattagcagagcgaggtatgtaggcggtgctacagagttcttgaagtggtggcctaactacggctacactagaaggacagtatttggtatctgcgctctgctgaagccagttaccttcggaaaaagagttggtagctcttgatccggcaaacaaaccaccgctggtagcggtggtttttttgtttgcaagcagcagattacgcgcagaaaaaaaggatctcaagaagatcctttgatcttttctacggggtctgacgctcagtggaacgaaaactcacgttaagggattttggtcatgagattatcaaaaaggatcttcacctagatccttttaaattaaaaatgaagttttaaatcaatctaaagtatatatgagtaaacttggtctgacagttaccaatgcttaatcagtgaggcacctatctcagcgatctgtctatttcgttcatccatagttgcctgactccccgtcgtgtagataactacgatacgggagggcttaccatctggccccagtgctgcaatgataccgcgagacccacgctcaccggctccagatttatcagcaataaaccagccagccggaagggccgagcgcagaagtggtcctgcaactttatccgcctccatccagtctattaattgttgccgggaagctagagtaagtagttcgccagttaatagtttgcgcaacgttgttgccattgctacaggcatcgtggtgtcacgctcgtcgtttggtatggcttcattcagctccggttcccaacgatcaaggcgagttacatgatcccccatgttgtgcaaaaaagcggttagctccttcggtcctccgatcgttgtcagaagtaagttggccgcagtgttatcactcatggttatggcagcactgcataattctcttactgtcatgccatccgtaagatgcttttctgtgactggtgagtactcaaccaagtcattctgagaatagtgtatgcggcgaccgagttgctcttgcccggcgtcaatacgggataataccgcgccacatagcagaactttaaaagtgctcatcattggaaaacgttcttcggggcgaaaactctcaaggatcttaccgctgttgagatccagttcgatgtaacccactcgtgcacccaactgatcttcagcatcttttactttcaccagcgtttctgggtgagcaaaaacaggaaggcaaaatgccgcaaaaaagggaataagggcgacacggaaatgttgaatactcatactcttcctttttcaatattattgaagcatttatcagggttattgtctcatgagcggatacatatttgaatgtatttagaaaaataaacaaataggggttccgcgcacatttccccgaaaagtgccac

SEQ ID NO: 8 - DNA, 2827 bp, Artificial Sequence
  Hsyn1:GGEDI-P2a-mApple
ctaaattgtaagcgttaatattttgttaaaattcgcgttaaatttttgttaaatcagctcattttttaaccaataggccgaaatcggcaaaatcccttataaatcaaaagaatagaccgagatagggttgagtgttgttccagtttggaacaagagtccactattaaagaacgtggactccaacgtcaaagggcgaaaaaccgtctatcagggcgatggcccactacgtgaaccatcaccctaatcaagttttttggggtcgaggtgccgtaaagcactaaatcggaaccctaaagggagcccccgatttagagcttgacggggaaagccggcgaacgtggcgagaaaggaagggaagaaagcgaaaggagcgggcgctagggcgctggcaagtgtagcggtcacgctgcgcgtaaccaccacacccgccgcgcttaatgcgccgctacagggcgcgtcccattcgccattcaggctgcgcaactgttgggaagggcgatcggtgcgggcctcttcgctattacgccagctggcgaaagggggatgtgctgcaaggcgattaagttgggtaacgccagggttttcccagtcacgacgttgtaaaacgacggccagtgagcgcgcgtaatacgactcactatagggcgaattgggtaccgccgccaccatgggtgacaatgacatccactttgcctttctctccacaggcgcgcactcccaggtccaactgcagggatccatggtcgactcttcacgtcgtaagtggaataagacaggtcacgcagtcagagctataggtcggctgagctcactcgagaacgtctatatcaaggccgacgagcagaagaacggcatcaaggcgtacttcaagatccgccacaacatcgagggcggcggcgtgcagctcgcctaccactaccagcagaacacccccatcggcgacggccccgtgctgctgcccgacaaccactacctgagcgtgcagtccatactttcgaaagaccccaacgagaagcgcgatcacatggtcctgctggagttcgtgaccgccgccgggatcactctcggcatggacgagctgtacaagggcggtaccggagggagcatggtgagcaagggcgaggagctgttcaccggggtggtgcccatccaggtcgagctggacggcgacgtaaacggccacaagttcagcgtgtccggcgagggtgagggcgatgccacctacggcaagctgaccctgaagttcatctgcaccaccggcaagctgcccgtgccctggcccaccctcgtgaccaccctgacctacggcgtgcagtgcttcagccgctaccccgaccacatgaagcagcacgacttcttcaagtccgccatgcccgaaggctacatccaggagcgcaccatcttcttcaaggacgacggcaactacaagacccgcgccgaggtgaagttcgagggcgacaccctggtgaaccgcatcgagctgaagggcatcgacttcaaggaggacggcaacatcctggggcacaagctggagtacaacacgcgtgaccaactgactgaagagcagatcgcagaatttaaagaggctttctccctatttgacaaggacggggatgggacgataacaaccaaggatctggggacggtgctgcggtctctggggcagaaccccacagaagcagagctccaggacatgatcaatgaagtagatgccgacggtaatggcacaatcgacttccctgagttcctgacaatgatggcaagaaaaatgaaagacacagacagtgaagaagaaattcgcgaagcgttccgtgtgtgggataaggatggcaatggctacatctctgcagcagaccttcgccacgtgatgacaaaccttggagagaagttaacagatgaagaggttgatgaaatgatcagggaagcagatatcgatggagaaggtcaggtaaactacgaagagtttgtacaaatgatgacagcgaaggcggccgcagaacaaaaactcatctcagaagaggatctgaatggggccgcaagcgagggatccggatccggagccacgaacttctctctgttaaagcaagcaggagacgtggaagaaaaccccggtcctatggtgagcaagggcgaggagaataacatggccatcatcaaggagttcatgcgcttcaaggtgcacatggagggctccgtgaacggccacgagttcgagatcgagggcgagggcgagggccgcccctacgaggcctttcagaccgctaagctgaaggtgaccaagggtggccccctgcccttcgcctgggacatcctgtcccctcagttcatgtacggctccaaggtctacattaagcacccagccgacatccccgactacttcaagctgtccttccccgagggcttcaggtgggagcgcgtgatgaacttcgaggacggcggcattattcacgttaaccaggactcctccctgcaggacggcgtgttcatctacaaggtgaagctgcgcggcaccaacttcccctccgacggccccgtaatgcagaagaagaccatgggctgggaggcctccgaggagcggatgtaccccgaggacggcgccctgaagagcgagatcaagaagaggctgaagctgaaggacggcggccactacgccgccgaggtcaagaccacctacaaggccaagaagcccgtgcagctgcccggcgcctacatcgtcgacatcaagttggacatcgtgtcccacaacgaggactacaccatcgtggaacagtacgaacgcgccgagggccgccactccaccggcggcatggacgagctgtacaagtaa

SEQ ID NO: 9 - DNA, 6756 bp, Artificial Sequence
  pAAV-hSyn1-mRuby2-GSG-P2A-GCaMP6f-WPRE-pA
ctgcagagggccctgcgtatgagtgcaagtgggttttaggaccaggatgaggcggggtgggggtgcctacctgacgaccgaccccgacccactggacaagcacccaacccccattccccaaattgcgcatcccctatcagagagggggaggggaaacaggatgcggcgaggcgcgtgcgcactgccagcttcagcaccgcggacagtgccttcgcccccgcctggcggcgcgcgccaccgccgcctcagcactgaaggcgcgctgacgtcactcgccggtcccccgcaaactccccttcccggccaccttggtcgcgtccgcgccgccgccggcccagccggaccgcaccacgcgaggcgcgagataggggggcacgggcgcgaccatctgcgctgcggcgccggcgactcagcgctgcctcagtctgcggtgggcagcggaggagtcgtgtcgtgcctgagagcgcagtcgaattcaagctgctagcaaggatccacccgccacctaccggtcctagggccaccatggtgtctaagggcgaagagctgatcaaggaaaatatgcgtatgaaggtggtcatggaaggttcggtcaacggccaccaattcaaatgcacaggtgaaggagaaggcaatccgtacatgggaactcaaaccatgaggatcaaagtcatcgagggaggacccctgccatttgcctttgacattcttgccacgtcgttcatgtatggcagccgtacttttatcaagtacccgaaaggcattcctgatttctttaaacagtcctttcctgagggttttacttgggaaagagttacgagatacgaagatggtggagtcgtcaccgtcatgcaggacaccagccttgaggatggctgtctcgtttaccacgtccaagtcagaggggtaaactttccctccaatggtcccgtgatgcagaagaagaccaagggttgggagcctaatacagagatgatgtatccagcagatggtggtctgaggggatacactcatatggcactgaaagttgatggtggtggccatctgtcttgctctttcgtaacaacttacaggtcaaaaaagaccgtcgggaacatcaagatgcccggtatccatgccgttgatcaccgcctggaaaggttagaggaaagtgacaatgaaatgttcgtagtacaacgcgaacacgcagttgccaagttcgccgggcttggtggtgggatggacgagctgtacaagggatccggagccacgaacttctctctgttaaagcaagcaggagacgtggaagaaaaccccggtcctggttctcatcatcatcatcatcatggtatggctagcatgactggtggacagcaaatgggtcgggatctgtacgacgatgacgataaggatctcgccaccatggtcgactcatcacgtcgtaagtggaataagacaggtcacgcagtcagagctataggtcggctgagctcactcgagaacgtctatatcaaggccgacaagcagaagaacggcatcaaggcgaacttcaagatccgccacaacatcgaggacggcggcgtgcagctcgcctaccactaccagcagaacacccccatcggcgacggccccgtgctgctgcccgacaaccactacctgagcgtgcagtccaaactttcgaaagaccccaacgagaagcgcgatcacatggtcctgctggagttcgtgaccgccgccgggatcactctcggcatggacgagctgtacaagggcggtaccggagggagcatggtgagcaagggcgaggagctgttcaccggggtggtgcccatcctggtcgagctggacggcgacgtaaacggccacaagttcagcgtgtccggcgagggtgagggcgatgccacctacggcaagctgaccctgaagttcatctgcaccaccggcaagctgcccgtgccctggcccaccctcgtgaccaccctgacctacggcgtgcagtgcttcagccgctaccccgaccacatgaagcagcacgacttcttcaagtccgccatgcccgaaggctacatccaggagcgcaccatcttcttcaaggacgacggcaactacaagacccgcgccgaggtgaagttcgagggcgacaccctggtgaaccgcatcgagctgaagggcatcgacttcaaggaggacggcaacatcctggggcacaagctggagtacaacctgccggaccaactgactgaagagcagatcgcagaatttaaagaggaattctccctatttgacaaggacggggatgggacaataacaaccaaggagctggggacggtgatgcggtctctggggcagaaccccacagaagcagagctgcaggacatgatcaatgaagtagatgccgacggtgacggcacaatcgacttccctgagttcctgacaatgatggcaagaaaaatgaaatacagggacacggaagaagaaattagagaagcgttcggtgtgtttgataaggatggcaatggctacatcagtgcagcagagcttcgccacgtgatgacaaaccttggagagaagttaacagatgaagaggttgatgaaatgatcagggaagcagacatcgatggggatggtcaggtaaactacgaagagtttgtacaaatgatgacagcgaagtaagcggccgcactagctagtgcggccgcttatgaaagctatcgataatcaacctctggattacaaaatttgtgaaagattgactggtattcttaactatgttgctccttttacgctatgtggatacgctgctttaatgcctttgtatcatgctattgcttcccgtatggctttcattttctcctccttgtataaatcctggttgctgtctctttatgaggagttgtggcccgttgtcaggcaacgtggcgtggtgtgcactgtgtttgctgacgcaacccccactggttggggcattgccaccacctgtcagctcctttccgggactttcgctttccccctccctattgccacggcggaactcatcgccgcctgccttgcccgctgctggacaggggctcggctgttgggcactgacaattccgtggtgttgtcggggaaatcatcgtcctttccttggctgctcgcctgtgttgccacctggattctgcgcgggacgtccttctgctacgtcccttcggccctcaatccagcggaccttccttcccgcggcctgctgccggctctgcggcctcttccgcgtcttcgccttcgccctcagacgagtcggatctccctttgggccgcctccccgcatcgataccgtcgacctcgacccgggcggccgcttcgagcagacatgataagatacattgatgagtttggacaaaccacaactagaatgcagtgaaaaaaatgctttatttgtgaaatttgtgatgctattgctttatttgtaaccattataagctgcaataaacaagttaacaacaacaattgcattcattttatgtttcaggttcagggggagatgtgggaggttttttaaagcaagtaaaacctctacaaatgtggtaaaatcgataaggatcttcctagagcatggctacgtagataagtagcatggcgggttaatcattaactacaaggaacccctagtgatggagttggccactccctctctgcgcgctcgctcgctcactgaggccgggcgaccaaaggtcgcccgacgcccgggctttgcccgggcggcctcagtgagcgagcgagcgcgcagccttaattaacctaattcactggccgtcgttttacaacgtcgtgactgggaaaaccctggcgttacccaacttaatcgccttgcagcacatccccctttcgccagctggcgtaatagcgaagaggcccgcaccgatcgcccttcccaacagttgcgcagcctgaatggcgaatgggacgcgccctgtagcggcgcattaagcgcggcgggtgtggtggttacgcgcagcgtgaccgctacacttgccagcgccctagcgcccgctcctttcgctttcttcccttcctttctcgccacgttcgccggctttccccgtcaagctctaaatcgggggctccctttagggttccgatttagtgctttacggcacctcgaccccaaaaaacttgattagggtgatggttcacgtagtgggccatcgccctgatagacggtttttcgccctttgacgttggagtccacgttctttaatagtggactcttgttccaaactggaacaacactcaaccctatctcggtctattcttttgatttataagggattttgccgatttcggcctattggttaaaaaatgagctgatttaacaaaaatttaacgcgaattttaacaaaatattaacgcttacaatttaggtggcacttttcggggaaatgtgcgcggaacccctatttgtttatttttctaaatacattcaaatatgtatccgctcatgagacaataaccctgataaatgcttcaataatattgaaaaaggaagagtatgagtattcaacatttccgtgtcgcccttattcccttttttgcggcattttgccttcctgtttttgctcacccagaaacgctggtgaaagtaaaagatgctgaagatcagttgggtgcacgagtgggttacatcgaactggatctcaacagcggtaagatccttgagagttttcgccccgaagaacgttttccaatgatgagcacttttaaagttctgctatgtggcgcggtattatcccgtattgacgccgggcaagagcaactcggtcgccgcatacactattctcagaatgacttggttgagtactcaccagtcacagaaaagcatcttacggatggcatgacagtaagagaattatgcagtgctgccataaccatgagtgataacactgcggccaacttacttctgacaacgatcggaggaccgaaggagctaaccgcttttttgcacaacatgggggatcatgtaactcgccttgatcgttgggaaccggagctgaatgaagccataccaaacgacgagcgtgacaccacgatgcctgtagcaatggcaacaacgttgcgcaaactattaactggcgaactacttactctagcttcccggcaacaattaatagactggatggaggcggataaagttgcaggaccacttctgcgctcggcccttccggctggctggtttattgctgataaatctggagccggtgagcgtgggtctcgcggtatcattgcagcactggggccagatggtaagccctcccgtatcgtagttatctacacgacggggagtcaggcaactatggatgaacgaaatagacagatcgctgagataggtgcctcactgattaagcattggtaactgtcagaccaagtttactcatatatactttagattgatttaaaacttcatttttaatttaaaaggatctaggtgaagatcctttttgataatctcatgaccaaaatcccttaacgtgagttttcgttccactgagcgtcagaccccgtagaaaagatcaaaggatcttcttgagatcctttttttctgcgcgtaatctgctgcttgcaaacaaaaaaaccaccgctaccagcggtggtttgtttgccggatcaagagctaccaactctttttccgaaggtaactggcttcagcagagcgcagataccaaatactgttcttctagtgtagccgtagttaggccaccacttcaagaactctgtagcaccgcctacatacctcgctctgctaatcctgttaccagtggctgctgccagtggcgataagtcgtgtcttaccgggttggactcaagacgatagttaccggataaggcgcagcggtcgggctgaacggggggttcgtgcacacagcccagcttggagcgaacgacctacaccgaactgagatacctacagcgtgagctatgagaaagcgccacgcttcccgaagggagaaaggcggacaggtatccggtaagcggcagggtcggaacaggagagcgcacgagggagcttccagggggaaacgcctggtatctttatagtcctgtcgggtttcgccacctctgacttgagcgtcgatttttgtgatgctcgtcaggggggcggagcctatggaaaaacgccagcaacgcggcctttttacggttcctggccttttgctggccttttgctcacatgttctttcctgcgttatcccctgattctgtggataaccgtattaccgcctttgagtgagctgataccgctcgccgcagccgaacgaccgagcgcagcgagtcagtgagcgaggaagcggaagagcgcccaatacgcaaaccgcctctccccgcgcgttggccgattcattaatgcagctggcacgacaggtttcccgactggaaagcgggcagtgagcgcaacgcaattaatgtgagttagctcactcattaggcaccccaggctttacactttatgcttccggctcgtatgttgtgtggaattgtgagcggataacaatttcacacaggaaacagctatgaccatgattacgccagatttaattaaggccttaattaggctgcgcgctcgctcgctcactgaggccgcccgggcaaagcccgggcgtcgggcgacctttggtcgcccggcctcagtgagcgagcgagcgcgcagagagggagtggccaactccatcactaggggttccttgtagttaatgattaacccgccatgctacttatctacgtagccatgctctaggaagatct

SEQ ID NO: 10 - DNA, 4324 bp, Artificial Sequence
  Hsyn1:RGEDI-P2a-3xTagBFP2
ctaaattgtaagcgttaatattttgttaaaattcgcgttaaatttttgttaaatcagctcattttttaaccaataggccgaaatcggcaaaatcccttataaatcaaaagaatagaccgagatagggttgagtgttgttccagtttggaacaagagtccactattaaagaacgtggactccaacgtcaaagggcgaaaaaccgtctatcagggcgatggcccactacgtgaaccatcaccctaatcaagttttttggggtcgaggtgccgtaaagcactaaatcggaaccctaaagggagcccccgatttagagcttgacggggaaagccggcgaacgtggcgagaaaggaagggaagaaagcgaaaggagcgggcgctagggcgctggcaagtgtagcggtcacgctgcgcgtaaccaccacacccgccgcgcttaatgcgccgctacagggcgcgtcccattcgccattcaggctgcgcaactgttgggaagggcgatcggtgcgggcctcttcgctattacgccagctggcgaaagggggatgtgctgcaaggcgattaagttgggtaacgccagggttttcccagtcacgacgttgtaaaacgacggccagtgagcgcgcgtaatacgactcactatagggcgaattgggtaccaagcttgccgccaccatgggtgacaatgacatccactttgcctttctctccacaggcgcgcactcccaggtccaactgcagggatccatggtcgactcttcacgtcgtaagtggaataaggcaggtcacgcagtcagagctataggtcggctgagctcacccgtggtttccgagcggatgtaccccgaggacggcgccctgaagagcgagatcaagaaggggctgaggctgaaggacggcggccactacgccgccgaggtcaagaccacctacaaggccaagaagcccgtgcagctgcccggcgcctacatcgtcgacatcaagttggacatcgtgtcccacaacgaggactacaccatcgtggaacagtgcgaacgcgccgagggccgccactccaccggcggcatggacgagctgtacaagggaggtacaggcgggagtctggtgagcaagggcgaggaggataacatggccatcatcaaggagttcatgcgcttcaaggtgcacatggagggctccgtgaacggccacgagttcgagatcgagggcgagggcgagggccgcccctacgaggcctttcagaccgctaagctgaaggtgaccaagggtggccccctgcccttcgcctgggacatcctgtcccctcagttcatgtacggctccaaggcctacattaagcacccagccgacatccccgactacttcaagctgtccttccccgagggcttcaggtgggagcgcgtgatgaacttcgaggacggcggcattattcacgttaaccaggactcctccctgcaggacggcgtattcatctacaaggtgaagctgcgcggcaccaacttcccccccgacggccccgtaatgcagaagaagaccatgggctgggaggctactcgagaccaactgactgaagagcagatcgcagaatttaaagaggctttctccctatttgacaaggacggggatgggacaataacaaccaaggatctggggacggtgctgcggtctctggggcagaaccccacagaagcagagctccaggacatgatcaatgaagtagatgccgacggtaatggcacaatcgacttccctgatttcctgacaatgatggcaagaaaaatgaaagacacagacagtgaagaagaaattcgcgaagcgttccgtgtgtgggataaggatggcaatggctacatctctgcagcagaccttcgccacgtgatgacaaaccttggagagaagttaacagatgaagaggttgatgaaatgatcagggaagcagatatcgatggagaaggtcaggtaaactacgaagagtttgtacaaatgatgacagcgaaggcggccgcagaacaaaaactcatctcagaagaggatctgaatggggccgcaagcgagggatccggatccggagccacgaacttctctctgttaaagcaagcaggagacgtggaagaaaaccccggtcctgggagccaccatcaccatcaccatggcagatctatgagcgagctgattaaggagaacatgcacatgaagctgtacatggagggcaccgtggacaaccatcacttcaagtgcacatccgagggcgaaggcaagccctacgagggcacccagaccatgagaatcaaggtggtcgagggcggccctctccccttcgccttcgacatcctggctactagcttcctctacggcagcaagaccttcatcaaccacacccagggcatccccgacttcttcaagcagtccttccctgagggcttcacatgggagagagtcaccacatacgaagacgggggcgtgctgaccgctacccaggacaccagcctccaggacggctgcctcatctacaacgtcaagatcagaggggtgaacttcacatccaacggccctgtgatgcagaagaaaacactcggctgggaggccttcaccgagacgctgtaccccgctgacggcggcctggaaggcagaaacgacatggccctgaagctcgtgggcgggagccatctgatcgcaaacgccaagaccacatatagatccaagaaacccgctaagaacctcaagatgcctggcgtctactatgtggactacagactggaaagaatcaaggaggccaacaacgagacctacgtcgagcagcacgaggtggcagtggccagatactgcgacctccctagcaaactggggcacaagcttaatgggagccaccatcaccatcaccatggcagatctatgagcgagctgattaaggagaacatgcacatgaagctgtacatggagggcaccgtggacaaccatcacttcaagtgcacatccgagggcgaaggcaagccctacgagggcacccagaccatgagaatcaaggtggtcgagggcggccctctccccttcgccttcgacatcctggctactagcttcctctacggcagcaagaccttcatcaaccacacccagggcatccccgacttcttcaagcagtccttccctgagggcttcacatgggagagagtcaccacatacgaagacgggggcgtgctgaccgctacccaggacaccagcctccaggacggctgcctcatctacaacgtcaagatcagaggggtgaacttcacatccaacggccctgtgatgcagaagaaaacactcggctgggaggccttcaccgagacgctgtaccccgctgacggcggcctggaaggcagaaacgacatggccctgaagctcgtgggcgggagccatctgatcgcaaacgccaagaccacatatagatccaagaaacccgctaagaacctcaagatgcctggcgtctactatgtggactacagactggaaagaatcaaggaggccaacaacgagacctacgtcgagcagcacgaggtggcagtggccagatactgcgacctccctagcaaactggggcacaagcttaatgggagccaccatcaccatcaccatggcagatctatgagcgagctgattaaggagaacatgcacatgaagctgtacatggagggcaccgtggacaaccatcacttcaagtgcacatccgagggcgaaggcaagccctacgagggcacccagaccatgagaatcaaggtggtcgagggcggccctctccccttcgccttcgacatcctggctactagcttcctctacggcagcaagaccttcatcaaccacacccagggcatccccgacttcttcaagcagtccttccctgagggcttcacatgggagagagtcaccacatacgaagacgggggcgtgctgaccgctacccaggacaccagcctccaggacggctgcctcatctacaacgtcaagatcagaggggtgaacttcacatccaacggccctgtgatgcagaagaaaacactcggctgggaggccttcaccgagacgctgtaccccgctgacggcggcctggaaggcagaaacgacatggccctgaagctcgtgggcgggagccatctgatcgcaaacgccaagaccacatatagatccaagaaacccgctaagaacctcaagatgcctggcgtctactatgtggactacagactggaaagaatcaaggaggccaacaacgagacctacgtcgagcagcacgaggtggcagtggccagatactgcgacctccctagcaaactggggcacaagcttaattaa

SEQ ID NO: 11 - DNA, 2881 bp, Artificial Sequence
  Hsyn1:RGEDInls-P2a-EGFPnls
ctaaattgtaagcgttaatattttgttaaaattcgcgttaaatttttgttaaatcagctcattttttaaccaataggccgaaatcggcaaaatcccttataaatcaaaagaatagaccgagatagggttgagtgttgttccagtttggaacaagagtccactattaaagaacgtggactccaacgtcaaagggcgaaaaaccgtctatcagggcgatggcccactacgtgaaccatcaccctaatcaagttttttggggtcgaggtgccgtaaagcactaaatcggaaccctaaagggagcccccgatttagagcttgacggggaaagccggcgaacgtggcgagaaaggaagggaagaaagcgaaaggagcgggcgctagggcgctggcaagtgtagcggtcacgctgcgcgtaaccaccacacccgccgcgcttaatgcgccgctacagggcgcgtcccattcgccattcaggctgcgcaactgttgggaagggcgatcggtgcgggcctcttcgctattacgccagctggcgaaagggggatgtgctgcaaggcgattaagttgggtaacgccagggttttcccagtcacgacgttgtaaaacgacggccagtgagcgcgcgtaatacgactcactatagggcgaattgggtaccaagcttgccgccaccatgggtgacaatgacatccactttgcctttctctccacaggcgcgcactcccaggtccaactgcagggatccatggtcgactcttcacgtcgtaagtggaataaggcaggtcacgcagtcagagctataggtcggctgagctcacccgtggtttccgagcggatgtaccccgaggacggcgccctgaagagcgagatcaagaaggggctgaggctgaaggacggcggccactacgccgccgaggtcaagaccacctacaaggccaagaagcccgtgcagctgcccggcgcctacatcgtcgacatcaagttggacatcgtgtcccacaacgaggactacaccatcgtggaacagtgcgaacgcgccgagggccgccactccaccggcggcatggacgagctgtacaagggaggtacaggcgggagtctggtgagcaagggcgaggaggataacatggccatcatcaaggagttcatgcgcttcaaggtgcacatggagggctccgtgaacggccacgagttcgagatcgagggcgagggcgagggccgcccctacgaggcctttcagaccgctaagctgaaggtgaccaagggtggccccctgcccttcgcctgggacatcctgtcccctcagttcatgtacggctccaaggcctacattaagcacccagccgacatccccgactacttcaagctgtccttccccgagggcttcaggtgggagcgcgtgatgaacttcgaggacggcggcattattcacgttaaccaggactcctccctgcaggacggcgtattcatctacaaggtgaagctgcgcggcaccaacttcccccccgacggccccgtaatgcagaagaagaccatgggctgggaggctactcgagaccaactgactgaagagcagatcgcagaatttaaagaggctttctccctatttgacaaggacggggatgggacaataacaaccaaggatctggggacggtgctgcggtctctggggcagaaccccacagaagcagagctccaggacatgatcaatgaagtagatgccgacggtaatggcacaatcgacttccctgatttcctgacaatgatggcaagaaaaatgaaagacacagacagtgaagaagaaattcgcgaagcgttccgtgtgtgggataaggatggcaatggctacatctctgcagcagaccttcgccacgtgatgacaaaccttggagagaagttaacagatgaagaggttgatgaaatgatcagggaagcagatatcgatggagaaggtcaggtaaactacgaagagtttgtacaaatgatgacagcgaaggcggccgcagaacaaaaactcatctcagaagaggatctgaatggggccgcaagcgagcaccttcctcttcttggatccggatccggagccacgaacttctctctgttaaagcaagcaggagacgtggaagaaaaccccggtcctatggtgagcaagggcgaggagctgttcaccggggtggtgcccatcctggtcgagctggacggcgacgtaaacggccacaagttcagcgtgtccggcgagggcgagggcgatgccacctacggcaagctgaccctgaagttcatctgcaccaccggcaagctgcccgtgccctggcccaccctcgtgaccaccctgacctacggcgtgcagtgcttcagccgctaccccgaccacatgaagcagcacgacttcttcaagtccgccatgcccgaaggctacgtccaggagcgcaccatcttcttcaaggacgacggcaactacaagacccgcgccgaggtgaagttcgagggcgacaccctggtgaaccgcatcgagctgaagggcatcgacttcaaggaggacggcaacatcctggggcacaagctggagtacaactacaacagccacaacgtctatatcatggccgacaagcagaagaacggcatcaaggtgaacttcaagatccgccacaacatcgaggacggcagcgtgcagctcgccgaccactaccagcagaacacccccatcggcgacggccccgtgctgctgcccgacaaccactacctgagcacccagtccgccctgagcaaagaccccaacgagaagcgcgatcacatggtcctgctggagttcgtgaccgccgccgggatcactctcggcatggacgagctgtacaagcaccttcctcttctttaaactagt

SEQ ID NO: 12 - DNA, 6876 bp, Artificial Sequence
  Hsyn1:GGEDI-P2a-jRCAMP1a
ctaaattgtaagcgttaatattttgttaaaattcgcgttaaatttttgttaaatcagctcattttttaaccaataggccgaaatcggcaaaatcccttataaatcaaaagaatagaccgagatagggttgagtgttgttccagtttggaacaagagtccactattaaagaacgtggactccaacgtcaaagggcgaaaaaccgtctatcagggcgatggcccactacgtgaaccatcaccctaatcaagttttttggggtcgaggtgccgtaaagcactaaatcggaaccctaaagggagcccccgatttagagcttgacggggaaagccggcgaacgtggcgagaaaggaagggaagaaagcgaaaggagcgggcgctagggcgctggcaagtgtagcggtcacgctgcgcgtaaccaccacacccgccgcgcttaatgcgccgctacagggcgcgtcccattcgccattcaggctgcgcaactgttgggaagggcgatcggtgcgggcctcttcgctattacgccagctggcgaaagggggatgtgctgcaaggcgattaagttgggtaacgccagggttttcccagtcacgacgttgtaaaacgacggccagtgagcgcgcgtaatacgactcactatagggcgaattgggtaccgggctgcagagggccctgcgtatgagtgcaagtgggttttaggaccaggatgaggcggggtgggggtgcctacctgacgaccgaccccgacccactggacaagcacccaacccccattccccaaattgcgcatcccctatcagagagggggaggggaaacaggatgcggcgaggcgcgtgcgcactgccagcttcagcaccgcggacagtgccttcgcccccgcctggcggcgcgcgccaccgccgcctcagcactgaaggcgcgctgacgtcactcgccggtcccccgcaaactccccttcccggccaccttggtcgcgtccgcgccgccgccggcccagccggaccgcaccacgcgaggcgcgagataggggggcacgggcgcgaccatctgcgctgcggcgccggcgactcagcgctgcctcagtctgcggtgggcagcggaggagtcgtgtcgtgcctgagagcgcagtcgaattcaagctgctagctagtaccggtcctagggccccccccctcgaggtcgacggtatcgataagcttgccgccaccatgggtgacaatgacatccactttgcctttctctccacaggcgcgcactcccaggtccaactgcagggatccatggtcgactcttcacgtcgtaagtggaataagacaggtcacgcagtcagagctataggtcggctgagctcactcgagaacgtctatatcaaggccgacgagcagaagaacggcatcaaggcgtacttcaagatccgccacaacatcgagggcggcggcgtgcagctcgcctaccactaccagcagaacacccccatcggcgacggccccgtgctgctgcccgacaaccactacctgagcgtgcagtccatactttcgaaagaccccaacgagaagcgcgatcacatggtcctgctggagttcgtgaccgccgccgggatcactctcggcatggacgagctgtacaagggcggtaccggagggagcatggtgagcaagggcgaggagctgttcaccggggtggtgcccatccaggtcgagctggacggcgacgtaaacggccacaagttcagcgtgtccggcgagggtgagggcgatgccacctacggcaagctgaccctgaagttcatctgcaccaccggcaagctgcccgtgccctggcccaccctcgtgaccaccctgacctacggcgtgcagtgcttcagccgctaccccgaccacatgaagcagcacgacttcttcaagtccgccatgcccgaaggctacatccaggagcgcaccatcttcttcaaggacgacggcaactacaagacccgcgccgaggtgaagttcgagggcgacaccctggtgaaccgcatcgagctgaagggcatcgacttcaaggaggacggcaacatcctggggcacaagctggagtacaacacgcgtgaccaactgactgaagagcagatcgcagaatttaaagaggctttctccctatttgacaaggacggggatgggacgataacaaccaaggatctggggacggtgctgcggtctctggggcagaaccccacagaagcagagctccaggacatgatcaatgaagtagatgccgacggtaatggcacaatcgacttccctgagttcctgacaatgatggcaagaaaaatgaaagacacagacagtgaagaagaaattcgcgaagcgttccgtgtgtgggataaggatggcaatggctacatctctgcagcagaccttcgccacgtgatgacaaaccttggagagaagttaacagatgaagaggttgatgaaatgatcagggaagcagatatcgatggagaaggtcaggtaaactacgaagagtttgtacaaatgatgacagcgaaggcggccgcagaacaaaaactcatctcagaagaggatctgaatggggccgcaagcgagggatccggatccggagccacgaacttctctctgttaaagcaagcaggagacgtggaagaaaaccccggtcctatgctgcagaacgagcttgctcttaagttggctggacttgatattaacaagactggaggaggttctcatcatcatcatcatcatggtatggctagcatgactggtggacagcaaatgggtcgggatctgtacgacgatgacgataaggatctcgcaacaatggtcgactcatcacgtcgtaagtggaataagacaggtcacgcagtcagagctataggtcggctgagctcagcgatcaactgcgaaatgatgtacccagcggatggtggtctgcgtggttacactcacatggcgctgaaagttgatggcggcggtcacctgtcctgttctttcgtgaccacctaccgctccaaaaagactgtcggcaacattaagatgcctgccattcatagcgtcagccaccgtctggagcgcctggaggagagcgataacgaaatgtttgtcgtacagcgtgaacacgcagttgccaagtttgtgggcctgggtggtggcggcggtaccggagggagcatgaactccctgatcaaggagaacatgcgtatgaaagtggttctggaaggctccgtaaacggccaccagttcaaatgcactggtgaaggcgaaggcaacccgtatatgggcacccagactatgcgtatcaaagtgatcgagggtggtccgctgccgtttgcgttcgacatcctggcgacgtcctttatgtatggctcccgtaccttcatcaaatatccgaaaggcatcccggatttctttaagcagtccttcccggaaggttttacctgggaacgtgtgacccgttacgaagacggcggcgtaattaccgttatgcaagacacgtctctggaggatggctgcctggtgtatcacgtgcaggttcgcggtgtgaacttcccgagcaatggtgctgtaatgcaaaagaaaaccaaaggttgggagcctacggactcccaaaccactgaagagcagatcgcagaatttaaagaggctttctccctatttgacaaggacggggatgggacaataacaaccaaggagctggggacggtgatgcggtctctggggcagaaccccacagaagcagagctgcaggacatgatcaatgaagtagatgccgacggtgacggcacaatcgacttccctgagttcctgattatgatggcaagaaaaatgaaatacacagacagtgaagaagaaattagagaagcgttcggcgtgtttgataaggatggcaatggctacatcagtgcagcagagcttcgccacgtgatgacaaaccttggagagaagttaacagatgaagaggttgatgaaatgatcagggaagcagacagcgatggggatggtcaggtaaactacgaagagtttgtacaaatgatgacagcgaagtagactagttctagagcggccgccaccgcggtgtcgataatcaacctctggattacaaaatttgtgaaagattgactggtattcttaactatgttgctccttttacgctatgtggatacgctgctttaatgcctttgtatcatgctattgcttcccgtatggctttcattttctcctccttgtataaatcctggttgctgtctctttatgaggagttgtggcccgttgtcaggcaacgtggcgtggtgtgcactgtgtttgctgacgcaacccccactggttggggcattgccaccacctgtcagctcctttccgggactttcgctttccccctccctattgccacggcggaactcatcgccgcctgccttgcccgctgctggacaggggctcggctgttgggcactgacaattccgtggtgttgtcggggaaatcatcgtcctttccttggctgctcgcctgtgttgccacctggattctgcgcgggacgtccttctgctacgtcccttcggccctcaatccagcggaccttccttcccgcggcctgctgccggctctgcggcctcttccgcgtcttcgccttcgccctcagacgagtcggatctccctttgggccgcctccccgcgagctccagcttttgttccctttagtgagggttaattgcgcgcttggcgtaatcatggtcatagctgtttcctgtgtgaaattgttatccgctcacaattccacacaacatacgagccggaagcataaagtgtaaagcctggggtgcctaatgagtgagctaactcacattaattgcgttgcgctcactgcccgctttccagtcgggaaacctgtcgtgccagctgcattaatgaatcggccaacgcgcggggagaggcggtttgcgtattgggcgctcttccgcttcctcgctcactgactcgctgcgctcggtcgttcggctgcggcgagcggtatcagctcactcaaaggcggtaatacggttatccacagaatcaggggataacgcaggaaagaacatgtgagcaaaaggccagcaaaaggccaggaaccgtaaaaaggccgcgttgctggcgtttttccataggctccgcccccctgacgagcatcacaaaaatcgacgctcaagtcagaggtggcgaaacccgacaggactataaagataccaggcgtttccccctggaagctccctcgtgcgctctcctgttccgaccctgccgcttaccggatacctgtccgcctttctcccttcgggaagcgtggcgctttctcatagctcacgctgtaggtatctcagttcggtgtaggtcgttcgctccaagctgggctgtgtgcacgaaccccccgttcagcccgaccgctgcgccttatccggtaactatcgtcttgagtccaacccggtaagacacgacttatcgccactggcagcagccactggtaacaggattagcagagcgaggtatgtaggcggtgctacagagttcttgaagtggtggcctaactacggctacactagaaggacagtatttggtatctgcgctctgctgaagccagttaccttcggaaaaagagttggtagctcttgatccggcaaacaaaccaccgctggtagcggtggtttttttgtttgcaagcagcagattacgcgcagaaaaaaaggatctcaagaagatcctttgatcttttctacggggtctgacgctcagtggaacgaaaactcacgttaagggattttggtcatgagattatcaaaaaggatcttcacctagatccttttaaattaaaaatgaagttttaaatcaatctaaagtatatatgagtaaacttggtctgacagttaccaatgcttaatcagtgaggcacctatctcagcgatctgtctatttcgttcatccatagttgcctgactccccgtcgtgtagataactacgatacgggagggcttaccatctggccccagtgctgcaatgataccgcgagacccacgctcaccggctccagatttatcagcaataaaccagccagccggaagggccgagcgcagaagtggtcctgcaactttatccgcctccatccagtctattaattgttgccgggaagctagagtaagtagttcgccagttaatagtttgcgcaacgttgttgccattgctacaggcatcgtggtgtcacgctcgtcgtttggtatggcttcattcagctccggttcccaacgatcaaggcgagttacatgatcccccatgttgtgcaaaaaagcggttagctccttcggtcctccgatcgttgtcagaagtaagttggccgcagtgttatcactcatggttatggcagcactgcataattctcttactgtcatgccatccgtaagatgcttttctgtgactggtgagtactcaaccaagtcattctgagaatagtgtatgcggcgaccgagttgctcttgcccggcgtcaatacgggataataccgcgccacatagcagaactttaaaagtgctcatcattggaaaacgttcttcggggcgaaaactctcaaggatcttaccgctgttgagatccagttcgatgtaacccactcgtgcacccaactgatcttcagcatcttttactttcaccagcgtttctgggtgagcaaaaacaggaaggcaaaatgccgcaaaaaagggaataagggcgacacggaaatgttgaatactcatactcttcctttttcaatattattgaagcatttatcagggttattgtctcatgagcggatacatatttgaatgtatttagaaaaataaacaaataggggttccgcgcacatttccccgaaaagtgccac